European Patent Application EP 4 151 654 A1, published March 22, 2023. Title: ST2 ANTIGEN BINDING PROTEIN. Applicant: Chia Tai Tianqing Pharmaceutical Group Co., Ltd. The sequence listing filed with the application follows.

SEQUENCE LISTING (86 sequences)

SEQ ID NO: 1 - protein, 556 aa, Homo sapiens
  UNSURE (78): X is E or A
MGFWILAILTILMYSTAAKFSKQSWGLENEALIVRCPRQGKPSYTVDWYYSQTNKSIPTQERNRVFASGQLLKFLPAXVADSGIYTCIVRSPTFNRTGYANVTIYKKQSDCNVPDYLMYSTVSGSEKNSKIYCPTIDLYNWTAPLEWFKNCQALQGSRYRAHKSFLVIDNVMTEDAGDYTCKFIHNENGANYSVTATRSFTVKDEQGFSLFPVIGAPAQNEIKEVEIGKNANLTCSACFGKGTQFLAAVLWQLNGTKITDFGEPRIQQEEGQNQSFSNGLACLDMVLRIADVKEEDLLLQYDCLALNLHGLRRHTVRLSRKNPIDHHSIYCIIAVCSVFLMLINVLVIILKMFWIEATLLWRDIAKPYKTRNDGKLYDAYVVYPRNYKSSTDGASRVEHFVHQILPDVLENKCGYTLCIYGRDMLPGEDVVTAVETNIRKSRRHIFILTPQITHNKEFAYEQEVALHCALIQNDAKVILIEMEALSELDMLQAEALQDSLQHLMKVQGTIKWREDHIANKRSLNSKFWKHVRYQMPVPSKIPRKASSLTPLAAQKQ

SEQ ID NO: 2 - protein, 566 aa, Artificial Sequence
  hST2-ECD-mFc
MGWSCIILFLVATGVHSKFSKQSWGLENEALIVRCPRQGKPSYTVDWYYSQTNKSIPTQERNRVFASGQLLKFLPAAVADSGIYTCIVRSPTFNRTGYANVTIYKKQSDCNVPDYLMYSTVSGSEKNSKIYCPTIDLYNWTAPLEWFKNCQALQGSRYRAHKSFLVIDNVMTEDAGDYTCKFIHNENGANYSVTATRSFTVKDEQGFSLFPVIGAPAQNEIKEVEIGKNANLTCSACFGKGTQFLAAVLWQLNGTKITDFGEPRIQQEEGQNQSFSNGLACLDMVLRIADVKEEDLLLQYDCLALNLHGLRRHTVRLSRKNPIDHHSIEGRMDEPRGPTIKPCPPCKCPAPNLLGGPSVFIFPPKIKDVLMISLSPIVTCVVVDVSEDDPDVQISWFVNNVEVHTAQTQTHREDYNSTLRVVSALPIQHQDWMSGKEFKCKVNNKDLPAPIERTISKPKGSVRAPQVYVLPPPEEEMTKKQVTLTCMVTDFMPEDIYVEWTNNGKTELNYKNTEPVLDSDGSYFMYSKLRVEKKNWVERNSYSCSVVHEGLHNHHTTKSFSRTPGK

SEQ ID NO: 3 - DNA, 1650 bp, Artificial Sequence
  hST2-ECD-mFc
aagttttctaagcagtcctggggcctggagaacgaggctctgatcgtgagatgtccccgccagggcaagcctagctacacagtggactggtactatagccagaccaacaagtctatcccaacacaggagagaaatcgcgtgttcgcctctggccagctgctgaagtttctgcccgccgctgtggctgatagcggcatctatacctgcatcgtgagatctcctaccttcaaccgcacaggctacgccaatgtgacaatctataagaagcagtccgactgtaacgtgcccgattacctgatgtattccaccgtgtccggcagcgagaagaatagcaagatctactgccctaccatcgacctgtataactggacagccccactggagtggttcaagaattgtcaggccctgcagggctctaggtaccgggctcacaagtccttcctggtcatcgataacgtgatgaccgaggacgctggcgattacacatgcaagttcatccataacgagaatggcgccaattattccgtgaccgctacaaggagctttacagtgaaggacgagcagggcttctccctgtttccagtgatcggcgcccccgctcagaacgagatcaaggaggtggagatcggcaagaacgccaatctgacctgctccgcctgtttcggcaagggcacacagtttctggccgctgtgctgtggcagctgaatggcaccaagatcacagatttcggcgagcctaggatccagcaggaggagggccagaaccagtctttttccaatggactggcttgcctggacatggtgctgaggatcgctgacgtgaaggaggaggatctgctgctgcagtatgattgtctggctctgaacctgcacggcctgaggcggcataccgtgaggctgtctcggaagaatccaatcgaccaccattccatcgagggaaggatggatgagccaaggggcccaaccatcaagccatgccccccttgcaagtgtcctgctccaaacctgctgggcggcccttccgtgttcatctttccacccaagatcaaggacgtgctgatgatctctctgtcccctatcgtgacatgcgtggtggtggacgtgtctgaggacgatccagatgtgcagatctcctggttcgtgaacaatgtggaggtgcacaccgcccagacccagacacatagggaggattacaattccacactgagggtggtgtccgccctgccaatccagcatcaggactggatgtccggcaaggagtttaagtgcaaggtgaacaataaggatctgcccgcccctatcgagaggaccatcagcaagcccaagggctctgtgcgggctcctcaggtgtatgtgctgcctccacccgaggaggagatgaccaagaagcaggtgaccctgacatgtatggtgacagacttcatgccagaggatatctacgtggagtggaccaacaatggcaagacagagctgaactataagaataccgagcccgtgctggactccgatggcagctactttatgtatagcaagctgagagtggagaagaagaactgggtggagcgcaatagctactcttgttccgtggtgcacgagggcctgcataaccaccataccacaaagagcttttctcggacacctggcaagtga

SEQ ID NO: 4 - protein, 565 aa, Artificial Sequence
  hST2-ECD-hFc
MGWSCIILFLVATGVHSKFSKQSWGLENEALIVRCPRQGKPSYTVDWYYSQTNKSIPTQERNRVFASGQLLKFLPAAVADSGIYTCIVRSPTFNRTGYANVTIYKKQSDCNVPDYLMYSTVSGSEKNSKIYCPTIDLYNWTAPLEWFKNCQALQGSRYRAHKSFLVIDNVMTEDAGDYTCKFIHNENGANYSVTATRSFTVKDEQGFSLFPVIGAPAQNEIKEVEIGKNANLTCSACFGKGTQFLAAVLWQLNGTKITDFGEPRIQQEEGQNQSFSNGLACLDMVLRIADVKEEDLLLQYDCLALNLHGLRRHTVRLSRKNPIDHHSIEGRMDEPKSCDKTHTCPPCPAPELLGGPSVFLFPPKPKDTLMISRTPEVTCVVVDVSHEDPEVKFNWYVDGVEVHNAKTKPREEQYNSTYRVVSVLTVLHQDWLNGKEYKCKVSNKALPAPIEKTISKAKGQPREPQVYTLPPSRDELTKNQVSLTCLVKGFYPSDIAVEWESNGQPENNYKTTPPVLDSDGSFFLYSKLTVDKSRWQQGNVFSCSVMHEALHNHYTQKSLSLSPGK

SEQ ID NO: 5 - DNA, 1647 bp, Artificial Sequence
  hST2-ECD-hFc
aagttttctaagcagtcctggggcctggagaacgaggctctgatcgtgagatgtccccgccagggcaagcctagctacacagtggactggtactatagccagaccaacaagtctatcccaacacaggagagaaatcgcgtgttcgcctctggccagctgctgaagtttctgcccgccgctgtggctgatagcggcatctatacctgcatcgtgagatctcctaccttcaaccgcacaggctacgccaatgtgacaatctataagaagcagtccgactgtaacgtgcccgattacctgatgtattccaccgtgtccggcagcgagaagaatagcaagatctactgccctaccatcgacctgtataactggacagccccactggagtggttcaagaattgtcaggccctgcagggctctaggtaccgggctcacaagtccttcctggtcatcgataacgtgatgaccgaggacgctggcgattacacatgcaagttcatccataacgagaatggcgccaattattccgtgaccgctacaaggagctttacagtgaaggacgagcagggcttctccctgtttccagtgatcggcgcccccgctcagaacgagatcaaggaggtggagatcggcaagaacgccaatctgacctgctccgcctgtttcggcaagggcacacagtttctggccgctgtgctgtggcagctgaatggcaccaagatcacagatttcggcgagcctaggatccagcaggaggagggccagaaccagtctttttccaatggactggcttgcctggacatggtgctgaggatcgctgacgtgaaggaggaggatctgctgctgcagtatgattgtctggctctgaacctgcacggcctgaggcggcataccgtgaggctgtctcggaagaatccaatcgaccaccattccatcgagggaaggatggatgagccaaagtcttgtgataagacccatacatgccccccttgtcctgctccagagctgctgggaggaccatccgtgttcctgtttccacccaagcccaaggacaccctgatgatctcccgcacaccagaggtgacctgcgtggtggtggacgtgagccacgaggatcccgaggtgaagtttaactggtacgtggatggcgtggaggtgcataatgctaagaccaagccaagagaggagcagtataacagcacataccgcgtggtgtctgtgctgaccgtgctgcaccaggactggctgaacggcaaggagtacaagtgcaaggtgtctaataaggccctgcccgctcctatcgagaagacaatctccaaggccaagggccagcctagggagccacaggtgtataccctgcctccatctcgggacgagctgacaaagaaccaggtgtccctgacctgtctggtgaagggcttctaccccagcgatatcgctgtggagtgggagtctaatggccagcctgagaacaattataagaccacaccccctgtgctggacagcgatggctctttctttctgtactctaagctgacagtggataagtccaggtggcagcagggcaacgtgtttagctgctctgtgatgcatgaggctctgcacaatcattacacccagaagtccctgagcctgtctcccggcaagtga

SEQ ID NO: 6 - protein, 174 aa, Artificial Sequence
  hIL33 Avitag
SITGISPITEYLASLSTYNDQSITFALEDESYEIYVEDLKKDEKKDKVLLSYYESQHPSNESGDGVDGKMLMVTLSPTKDFWLHANNKEHSVELHKCEKPLPDQAFFVLHNMHSNCVSFECKTDPGVFIGVKDNHLALIKVDSSENLCTENILFKLSETGLNDIFEAQKIEWHE

SEQ ID NO: 7 - DNA, 525 bp, Artificial Sequence
  hIL33 Avitag
agcataacaggaatatcacccataactgaatatctagcttcattaagtacatataacgatcagagcattaccttcgcgctggaggacgaaagctacgagatctatgtggaagacctgaagaaagatgaaaagaaagacaaggttctgctgagctactatgagagccaacacccgagcaacgaaagcggtgacggcgtggatggcaaaatgctgatggttaccctgagcccgaccaaggacttttggctgcacgcgaacaacaaagagcacagcgtggaactgcacaagtgcgagaaaccgctgccggatcaggcgttctttgtgctgcacaacatgcacagcaactgcgttagcttcgaatgcaagaccgatccgggtgtgtttattggcgttaaggacaaccacctggcgctgatcaaagttgatagcagcgagaacctgtgcaccgaaaacattctgttcaagctgagcgagaccggtctgaacgacatttttgaagcgcaaaaaatcgagtggcacgaataa

SEQ ID NO: 8 - protein, 159 aa, Artificial Sequence
  hIL33 protein
SITGISPITEYLASLSTYNDQSITFALEDESYEIYVEDLKKDEKKDKVLLSYYESQHPSNESGDGVDGKMLMVTLSPTKDFWLHANNKEHSVELHKCEKPLPDQAFFVLHNMHSNCVSFECKTDPGVFIGVKDNHLALIKVDSSENLCTENILFKLSET

SEQ ID NO: 9 - DNA, 477 bp, Artificial Sequence
  hIL33 protein
agcataacaggaatatcacccataactgaatatctagcttcattaagtacatataacgatcagagcattaccttcgcgctggaggacgaaagctacgagatctatgtggaagacctgaagaaagatgaaaagaaagacaaggttctgctgagctactatgagagccaacacccgagcaacgaaagcggtgacggcgtggatggcaaaatgctgatggttaccctgagcccgaccaaggacttttggctgcacgcgaacaacaaagagcacagcgtggaactgcacaagtgcgagaaaccgctgccggatcaggcgttctttgtgctgcacaacatgcacagcaactgcgttagcttcgaatgcaagaccgatccgggtgtgtttattggcgttaaggacaaccacctggcgctgatcaaagttgatagcagcgagaacctgtgcaccgaaaacattctgttcaagctgagcgagacc

SEQ ID NO: 10 - protein, 556 aa, Cynomolgus monkey (Macaca fascicularis)
MGLWILAILTILVYSTAAKFSKQSWGLENEALIVRCPRQGKSSYIVDWYYSQTNKSIPTQERNRVFASGQLLKFLPAEVADSGIYTCIVRSPTFNRTGYANVTIYKKQPDCNVPDYLMYSTVSGSEKNSKIYCPTIDLYNWTAPLEWFKNCQALQGSRYKAHKSFLVIDNVMTDDAGDYTCKFIHNENGANYSVTATRSFTVKDEQGFSRFPVIRAPAHNETKEVEIGENTNLTCSACFGKGAQFLAAVQWQLNGNKITDFSEPRIQQEEGQNQSFSDGLACVNTVLRIADVKEEDLLLRYDCLALNLHGLRRHTIRLSRKNPIDHQSTYCIIAVCSVLLMLINVLVIILKTFWIEATLLWRDIAKPYKTRNDGKLYDAYVIYPRNYTSSTDGASRVEYFVHQILPDVLENKCGYTLCIYGRDMLPGEDVVTAVETNIRKSRRHIFILTPQITHSEEFAYEQEVALHSALIQNDSKVILIEMEALSELDMLQAEALQDSLRHLMEVQGTIKWREDHVANKRSLNSKFWKHVRYQMPVPSKMPRKASSLTSLAAQKQ

SEQ ID NO: 11 - protein, 5 aa, Mouse (Mus sp.)
DYEMH

SEQ ID NO: 12 - protein, 5 aa, Mouse (Mus sp.)
DSEMH

SEQ ID NO: 13 - protein, 5 aa, Mouse (Mus sp.)
DSEIH

SEQ ID NO: 14 - protein, 5 aa, Mouse (Mus sp.)
DYEMQ

SEQ ID NO: 15 - protein, 17 aa, Mouse (Mus sp.)
TIDPETGDTAYNQKFKG

SEQ ID NO: 16 - protein, 17 aa, Mouse (Mus sp.)
AIDPETGDTAYSQNFKG

SEQ ID NO: 17 - protein, 17 aa, Artificial Sequence
  UNSURE (12): X is N or A
  UNSURE (13): X is Q or E or K
  UNSURE (16): X is K or Q
  HV-CDR2 of antibody 31C8
AIDPETGDTVYXXKFXG

SEQ ID NO: 18 - protein, 17 aa, Mouse (Mus sp.)
AIDPETGDTAYNQKFKG

SEQ ID NO: 19 - protein, 17 aa, Mouse (Mus sp.)
AFDPETGDTAYNQKFKG

SEQ ID NO: 20 - protein, 12 aa, Mouse (Mus sp.)
YSYTNSPYGMDY

SEQ ID NO: 21 - protein, 9 aa, Mouse (Mus sp.)
SATDYYFAS

SEQ ID NO: 22 - protein, 9 aa, Mouse (Mus sp.)
STTDYYFAY

SEQ ID NO: 23 - protein, 9 aa, Mouse (Mus sp.)
STTDCYFAY

SEQ ID NO: 24 - protein, 10 aa, Mouse (Mus sp.)
VDSNYDYFDY

SEQ ID NO: 25 - protein, 11 aa, Mouse (Mus sp.)
KASQSVSNDVA

SEQ ID NO: 26 - protein, 16 aa, Mouse (Mus sp.)
RSSKSLLHSNGITYLY

SEQ ID NO: 27 - protein, 16 aa, Mouse (Mus sp.)
RSSKSLLHSNGIIYLY

SEQ ID NO: 28 - protein, 10 aa, Mouse (Mus sp.)
RASSSVSYMH

SEQ ID NO: 29 - protein, 7 aa, Mouse (Mus sp.)
YASNRYT

SEQ ID NO: 30 - protein, 7 aa, Artificial Sequence
  UNSURE (2): X is M or L
  LV-CDR2s of antibodies 3C6, 31C8, 26A1 and 8F4
QXSNLAS

SEQ ID NO: 31 - protein, 7 aa, Mouse (Mus sp.)
DTSNLAS

SEQ ID NO: 32 - protein, 9 aa, Mouse (Mus sp.)
QQDYSSPYT

SEQ ID NO: 33 - protein, 9 aa, Mouse (Mus sp.)
QQWSSNPLT

SEQ ID NO: 34 - protein, 9 aa, Mouse (Mus sp.)
AQNLELPFT

SEQ ID NO: 35 - protein, 121 aa, Mouse (Mus sp.)
QVQLQQSGAELVRPGASVTLSCKASGYTFTDYEMHWVKQTPVHGLDWIGTIDPETGDTAYNQKFKGRATLTADKSSSTAYMELSSLTSEDSAVYYCTRYSYTNSPYGMDYWGQGTSVTVSS

SEQ ID NO: 36 - protein, 107 aa, Mouse (Mus sp.)
DVVMTQTPKFLLVSAGDRVTITCKASQSVSNDVAWYQQKPGQSPKLLIYYASNRYTGVPDRFTGSGYGTDFTFTINTVQAEDLAVYFCQQDYSSPYTFGGGTKLEIK

SEQ ID NO: 37 - protein, 118 aa, Mouse (Mus sp.)
QVQLQQSGAEVVRPGASVTLSCKASDYTITDYEMHWVKQTPVHGLEWIGAIDPETGDTAYSQNFKGKATLTADESSSTAYMELSSLTSEDSAVYYCSRSATDYYFASWGQGTTLTVSS

SEQ ID NO: 38 - protein, 112 aa, Mouse (Mus sp.)
DIVMTQAAISNPVTLGTSASMSCRSSKSLLHSNGITYLYWYLQKPGHSPQLLIYQMSNLASGVPDRFSSSGSGTDFTLKISRVEAEDVGVYYCAQNLELPFTFGSGTKLEIK

SEQ ID NO: 39 - protein, 118 aa, Mouse (Mus sp.)
QVQLQQSGPELVRPGASVTLSCKASGYIFIDSEMHWVKQTPVHGLEWIGAIDPETGDTVYNQKFKGKATLTADKSSSTASMELSSLTSEDSAVYYCTGSTTDYYFAYWGQGTTLTVSS

SEQ ID NO: 40 - protein, 112 aa, Mouse (Mus sp.)
DIVMTQAAFSNPVTLGTSASISCRSSKSLLHSNGIIYLYWYLQKPGQSPQLLIYQMSNLASGVPDRFSSSGSGTDFTLRISRVEAEDVGVYYCAQNLELPFTFGSGTKLEIK

SEQ ID NO: 41 - protein, 118 aa, Mouse (Mus sp.)
QVQLQQSGAELVRPGASVTLSCKASDYIFTDSEIHWVKQTLVHGLEWIGAIDPETGDTAYNQKFKGKATLTADKSSSTAYMELSSLTSEGSAVYYCSGSTTDCYFAYWGQGTTLTVSS

SEQ ID NO: 42 - protein, 112 aa, Mouse (Mus sp.); identical to SEQ ID NO: 40

SEQ ID NO: 43 - protein, 118 aa, Mouse (Mus sp.)
QVQLQQSGAELVRPGASVTLSCKASGHIFTDYEMQWVKQTPVHGLEWIGAFDPETGDTAYNQKFKGKATLTADKSSSTAYMELSSLTSEDSAVYYCSGSTTDYYFAYWGQGTSLTVSS

SEQ ID NO: 44 - protein, 112 aa, Mouse (Mus sp.)
DVVMTQTAFSNPVTLGTSASISCRSSKSLLHSNGIIYLYWYLQKPGQSPQLLIYQMSNLASGVPDRFSSSGSGTDFTLRISRVEAEDVGVYYCAQNLELPFTFGSGTKLEIK

SEQ ID NO: 45 - protein, 119 aa, Mouse (Mus sp.)
QVQLQQSGAELVRPGASVTLSCKASGYTFTDYEMHWVKQTPVLGLEWIGAIDPETGDTAYNQKFKGKATLTADKSSSTAYMELSSLASEDSAVYYCIRVDSNYDYFDYWGQDTTLTVSS

SEQ ID NO: 46 - protein, 106 aa, Mouse (Mus sp.)
DIVLTQSPPILSASPGEKVTMTCRASSSVSYMHWYQQKPGSSPKPWIYDTSNLASGVPARFSGSGSGTSYSLTISRVEAEDAATYYCQQWSSNPLTFGAGTKLELK

SEQ ID NO: 47 - protein, 447 aa, Artificial Sequence
  Heavy chain of chimeric antibody 7D1
QVQLQQSGAELVRPGASVTLSCKASGYTFTDYEMHWVKQTPVHGLDWIGTIDPETGDTAYNQKFKGRATLTADKSSSTAYMELSSLTSEDSAVYYCTRYSYTNSPYGMDYWGQGTSVTVSSASTKGPSVFPLAPCSRSTSESTAALGCLVKDYFPEPVTVSWNSGALTSGVHTFPAVLQSSGLYSLSSVVTVPSSNFGTQTYTCNVDHKPSNTKVDKTVERKCCVECPPCPAPPVAGPSVFLFPPKPKDTLMISRTPEVTCVVVDVSHEDPEVQFNWYVDGVEVHNAKTKPREEQFNSTFRVVSVLTVVHQDWLNGKEYKCKVSNKGLPAPIEKTISKTKGQPREPQVYTLPPSREEMTKNQVSLTCLVKGFYPSDISVEWESNGQPENNYKTTPPMLDSDGSFFLYSKLTVDKSRWQQGNVFSCSVMHEALHNHYTQKSLSLSPGK

SEQ ID NO: 48 - DNA, 1344 bp, Artificial Sequence
  Heavy chain of chimeric antibody 7D1
caggtgcagctgcagcagtctggagctgagctggtgaggccaggagcttccgtgaccctgagctgcaaggcctctggctacaccttcacagactatgagatgcactgggtgaagcagacccccgtgcatggcctggattggatcggcacaatcgaccctgagaccggcgatacagcttacaaccagaagtttaagggcagggccaccctgacagctgacaagtccagctctaccgcctatatggagctgtccagcctgacaagcgaggattccgccgtgtactattgtacccggtactcctatacaaatagcccctacggcatggactattggggccagggcacctccgtgacagtgtcttccgctagcacaaagggccctagcgtgttcccactggctccctgctccagaagcacatctgagtccaccgccgctctgggctgtctggtgaaggactacttccctgagccagtgacagtgtcctggaacagcggcgccctgacatccggagtgcacacctttccagctgtgctgcagtccagcggcctgtacagcctgtcttccgtggtgaccgtgcccagctctaattttggcacccagacatatacctgcaacgtggaccataagccttctaatacaaaggtggataagaccgtggagaggaagtgctgcgtggagtgcccaccttgtccagctccaccagtggctggcccttccgtgttcctgtttcctccaaagccaaaggacacactgatgatctctcggacacccgaggtgacctgcgtggtggtggacgtgtcccacgaggatccagaggtgcagttcaactggtacgtggatggcgtggaggtgcataatgccaagaccaagcccagggaggagcagttcaactctacatttcgggtggtgtccgtgctgaccgtggtgcaccaggattggctgaacggcaaggagtataagtgcaaggtgagcaataagggcctgcccgctcctatcgagaagacaatctctaagaccaagggccagcctagagagccacaggtgtacaccctgcccccttcccgcgaggagatgacaaagaaccaggtgagcctgacctgtctggtgaagggcttctatccttctgacatctccgtggagtgggagagcaatggccagccagagaacaattacaagaccacaccacccatgctggacagcgatggctctttctttctgtatagcaagctgacagtggataagtctcgctggcagcagggcaacgtgtttagctgctctgtgatgcatgaggccctgcacaatcattatacccagaagtccctgagcctgtctcccggcaagtga

SEQ ID NO: 49 - protein, 214 aa, Artificial Sequence
  Light chain of chimeric antibody 7D1
DVVMTQTPKFLLVSAGDRVTITCKASQSVSNDVAWYQQKPGQSPKLLIYYASNRYTGVPDRFTGSGYGTDFTFTINTVQAEDLAVYFCQQDYSSPYTFGGGTKLEIKRTVAAPSVFIFPPSDEQLKSGTASVVCLLNNFYPREAKVQWKVDNALQSGNSQESVTEQDSKDSTYSLSSTLTLSKADYEKHKVYACEVTHQGLSSPVTKSFNRGEC

SEQ ID NO: 50 - DNA, 645 bp, Artificial Sequence
  Light chain of chimeric antibody 7D1
gacgtggtcatgacccagacacccaagttcctgctggtgagcgccggcgacagggtgaccatcacatgcaaggcctctcagtccgtgagcaacgatgtggcttggtaccagcagaagcccggccagtctcctaagctgctgatctactatgcttccaataggtacaccggcgtgccagaccggtttaccggctctggctatggcacagatttcacctttacaatcaacacagtgcaggccgaggacctggccgtgtacttctgtcagcaggattactccagcccctatacctttggcggcggcacaaagctggagatcaagcgtacggtggccgctcccagcgtgttcatctttcccccttctgacgagcagctgaagtctggcaccgcttccgtggtgtgcctgctgaacaatttctaccccagagaggccaaggtgcagtggaaggtggataacgctctgcagtccggcaatagccaggagtctgtgaccgagcaggactccaaggatagcacatattctctgtcttccaccctgacactgtctaaggccgactacgagaagcacaaggtgtatgcttgcgaggtgacccatcagggcctgagctctcctgtgacaaagtcctttaatcgcggcgagtgttga

SEQ ID NO: 51 - protein, 444 aa, Artificial Sequence
  Heavy chain of chimeric antibody 3C6
QVQLQQSGAEVVRPGASVTLSCKASDYTITDYEMHWVKQTPVHGLEWIGAIDPETGDTAYSQNFKGKATLTADESSSTAYMELSSLTSEDSAVYYCSRSATDYYFASWGQGTTLTVSSASTKGPSVFPLAPCSRSTSESTAALGCLVKDYFPEPVTVSWNSGALTSGVHTFPAVLQSSGLYSLSSVVTVPSSNFGTQTYTCNVDHKPSNTKVDKTVERKCCVECPPCPAPPVAGPSVFLFPPKPKDTLMISRTPEVTCVVVDVSHEDPEVQFNWYVDGVEVHNAKTKPREEQFNSTFRVVSVLTVVHQDWLNGKEYKCKVSNKGLPAPIEKTISKTKGQPREPQVYTLPPSREEMTKNQVSLTCLVKGFYPSDISVEWESNGQPENNYKTTPPMLDSDGSFFLYSKLTVDKSRWQQGNVFSCSVMHEALHNHYTQKSLSLSPGK

SEQ ID NO: 52 - DNA, 1344 bp, Artificial Sequence; identical to SEQ ID NO: 48
  Heavy chain of chimeric antibody 3C6

SEQ ID NO: 53 - protein, 219 aa, Artificial Sequence
  Light chain of chimeric antibody 3C6
DIVMTQAAISNPVTLGTSASMSCRSSKSLLHSNGITYLYWYLQKPGHSPQLLIYQMSNLASGVPDRFSSSGSGTDFTLKISRVEAEDVGVYYCAQNLELPFTFGSGTKLEIKRTVAAPSVFIFPPSDEQLKSGTASVVCLLNNFYPREAKVQWKVDNALQSGNSQESVTEQDSKDSTYSLSSTLTLSKADYEKHKVYACEVTHQGLSSPVTKSFNRGEC

SEQ ID NO: 54 - DNA, 660 bp, Artificial Sequence
  Light chain of chimeric antibody 3C6
gacatcgtgatgacccaggccgctatctctaaccccgtgaccctgggcacatctgcctccatgagctgcaggtccagcaagtctctgctgcactccaatggcatcacatacctgtattggtacctgcagaagcccggccattcccctcagctgctgatctatcagatgagcaacctggcttctggcgtgccagacaggttctcttccagcggctccggcaccgacttcaccctgaagatcagcagggtggaggctgaggatgtgggcgtgtactattgtgctcagaatctggagctgcccttcacctttggctccggcacaaagctggagatcaagcgtacggtggccgctcccagcgtgttcatctttcccccttctgacgagcagctgaagtctggcaccgcttccgtggtgtgcctgctgaacaatttctaccccagagaggccaaggtgcagtggaaggtggataacgctctgcagtccggcaatagccaggagtctgtgaccgagcaggactccaaggatagcacatattctctgtcttccaccctgacactgtctaaggccgactacgagaagcacaaggtgtatgcttgcgaggtgacccatcagggcctgagctctcctgtgacaaagtcctttaatcgcggcgagtgttga

SEQ ID NO: 55 - protein, 444 aa, Artificial Sequence
  Heavy chain of chimeric antibody 26A1
QVQLQQSGAELVRPGASVTLSCKASDYIFTDSEIHWVKQTLVHGLEWIGAIDPETGDTAYNQKFKGKATLTADKSSSTAYMELSSLTSEGSAVYYCSGSTTDCYFAYWGQGTTLTVSSASTKGPSVFPLAPCSRSTSESTAALGCLVKDYFPEPVTVSWNSGALTSGVHTFPAVLQSSGLYSLSSVVTVPSSNFGTQTYTCNVDHKPSNTKVDKTVERKCCVECPPCPAPPVAGPSVFLFPPKPKDTLMISRTPEVTCVVVDVSHEDPEVQFNWYVDGVEVHNAKTKPREEQFNSTFRVVSVLTVVHQDWLNGKEYKCKVSNKGLPAPIEKTISKTKGQPREPQVYTLPPSREEMTKNQVSLTCLVKGFYPSDISVEWESNGQPENNYKTTPPMLDSDGSFFLYSKLTVDKSRWQQGNVFSCSVMHEALHNHYTQKSLSLSPGK

SEQ ID NO: 56 - DNA, 1335 bp, Artificial Sequence
  Heavy chain of chimeric antibody 26A1
caggtgcagctgcagcagtctggagctgagctggtgaggccaggagcttctgtgaccctgtcctgcaaggccagcgactacatcttcaccgattccgagatccactgggtgaagcagacactggtgcatggcctggagtggatcggagctatcgaccctgagaccggcgatacagcttacaaccagaagtttaagggcaaggccaccctgacagctgacaagtccagctctaccgcctatatggagctgtccagcctgacatccgagggctccgccgtgtactattgcagcggctctaccacagattgttacttcgcttattggggccagggcaccacactgacagtgtcttccgctagcacaaagggccctagcgtgttcccactggctccctgctccagaagcacatctgagtccaccgccgctctgggctgtctggtgaaggactacttccctgagccagtgacagtgtcctggaacagcggcgccctgacatccggagtgcacacctttccagctgtgctgcagtccagcggcctgtacagcctgtcttccgtggtgaccgtgcccagctctaattttggcacccagacatatacctgcaacgtggaccataagccttctaatacaaaggtggataagaccgtggagaggaagtgctgcgtggagtgcccaccttgtccagctccaccagtggctggcccttccgtgttcctgtttcctccaaagccaaaggacacactgatgatctctcggacacccgaggtgacctgcgtggtggtggacgtgtcccacgaggatccagaggtgcagttcaactggtacgtggatggcgtggaggtgcataatgccaagaccaagcccagggaggagcagttcaactctacatttcgggtggtgtccgtgctgaccgtggtgcaccaggattggctgaacggcaaggagtataagtgcaaggtgagcaataagggcctgcccgctcctatcgagaagacaatctctaagaccaagggccagcctagagagccacaggtgtacaccctgcccccttcccgcgaggagatgacaaagaaccaggtgagcctgacctgtctggtgaagggcttctatccttctgacatctccgtggagtgggagagcaatggccagccagagaacaattacaagaccacaccacccatgctggacagcgatggctctttctttctgtatagcaagctgacagtggataagtctcgctggcagcagggcaacgtgtttagctgctctgtgatgcatgaggccctgcacaatcattatacccagaagtccctgagcctgtctcccggcaagtga

SEQ ID NO: 57 - protein, 219 aa, Artificial Sequence
  Light chain of chimeric antibody 26A1
DIVMTQAAFSNPVTLGTSASISCRSSKSLLHSNGIIYLYWYLQKPGQSPQLLIYQMSNLASGVPDRFSSSGSGTDFTLRISRVEAEDVGVYYCAQNLELPFTFGSGTKLEIKRTVAAPSVFIFPPSDEQLKSGTASVVCLLNNFYPREAKVQWKVDNALQSGNSQESVTEQDSKDSTYSLSSTLTLSKADYEKHKVYACEVTHQGLSSPVTKSFNRGEC

SEQ ID NO: 58 - DNA, 660 bp, Artificial Sequence
  Light chain of chimeric antibody 26A1
gacatcgtgatgacccaggccgctttctctaaccccgtgaccctgggcacatctgcctccatcagctgcagatccagcaagtctctgctgcactccaatggcatcatctacctgtattggtacctgcagaagcccggccagtcccctcagctgctgatctatcagatgagcaacctggcttctggcgtgccagaccgcttctcttccagcggctccggcaccgacttcaccctgaggatcagcagggtggaggctgaggatgtgggcgtgtactattgtgctcagaatctggagctgcccttcacctttggctccggcacaaagctggagatcaagcgtacggtggccgctcccagcgtgttcatctttcccccttctgacgagcagctgaagtctggcaccgcttccgtggtgtgcctgctgaacaatttctaccccagagaggccaaggtgcagtggaaggtggataacgctctgcagtccggcaatagccaggagtctgtgaccgagcaggactccaaggatagcacatattctctgtcttccaccctgacactgtctaaggccgactacgagaagcacaaggtgtatgcttgcgaggtgacccatcagggcctgagctctcctgtgacaaagtcctttaatcgcggcgagtgttga

SEQ ID NO: 59 - protein, 444 aa, Artificial Sequence
  Heavy chain of chimeric antibody 8F4
QVQLQQSGAELVRPGASVTLSCKASGHIFTDYEMQWVKQTPVHGLEWIGAFDPETGDTAYNQKFKGKATLTADKSSSTAYMELSSLTSEDSAVYYCSGSTTDYYFAYWGQGTSLTVSSASTKGPSVFPLAPCSRSTSESTAALGCLVKDYFPEPVTVSWNSGALTSGVHTFPAVLQSSGLYSLSSVVTVPSSNFGTQTYTCNVDHKPSNTKVDKTVERKCCVECPPCPAPPVAGPSVFLFPPKPKDTLMISRTPEVTCVVVDVSHEDPEVQFNWYVDGVEVHNAKTKPREEQFNSTFRVVSVLTVVHQDWLNGKEYKCKVSNKGLPAPIEKTISKTKGQPREPQVYTLPPSREEMTKNQVSLTCLVKGFYPSDISVEWESNGQPENNYKTTPPMLDSDGSFFLYSKLTVDKSRWQQGNVFSCSVMHEALHNHYTQKSLSLSPGK

SEQ ID NO: 60 - DNA, 1335 bp, Artificial Sequence
  Heavy chain of chimeric antibody 8F4
caggtgcagctgcagcagtctggagctgagctggtgaggccaggagcttctgtgaccctgtcctgcaaggccagcggccacatcttcaccgactacgagatgcagtgggtgaagcagacaccagtgcatggactggagtggatcggagccttcgaccctgagaccggcgatacagcttacaaccagaagtttaagggcaaggccaccctgacagctgataagtccagctctaccgcctatatggagctgtccagcctgacatccgaggactccgccgtgtactattgtagcggctctaccacagattactattttgcttattggggccagggcacctccctgacagtgtcttccgctagcacaaagggccctagcgtgttcccactggctccctgctccagaagcacatctgagtccaccgccgctctgggctgtctggtgaaggactacttccctgagccagtgacagtgtcctggaacagcggcgccctgacatccggagtgcacacctttccagctgtgctgcagtccagcggcctgtacagcctgtcttccgtggtgaccgtgcccagctctaattttggcacccagacatatacctgcaacgtggaccataagccttctaatacaaaggtggataagaccgtggagaggaagtgctgcgtggagtgcccaccttgtccagctccaccagtggctggcccttccgtgttcctgtttcctccaaagccaaaggacacactgatgatctctcggacacccgaggtgacctgcgtggtggtggacgtgtcccacgaggatccagaggtgcagttcaactggtacgtggatggcgtggaggtgcataatgccaagaccaagcccagggaggagcagttcaactctacatttcgggtggtgtccgtgctgaccgtggtgcaccaggattggctgaacggcaaggagtataagtgcaaggtgagcaataagggcctgcccgctcctatcgagaagacaatctctaagaccaagggccagcctagagagccacaggtgtacaccctgcccccttcccgcgaggagatgacaaagaaccaggtgagcctgacctgtctggtgaagggcttctatccttctgacatctccgtggagtgggagagcaatggccagccagagaacaattacaagaccacaccacccatgctggacagcgatggctctttctttctgtatagcaagctgacagtggataagtctcgctggcagcagggcaacgtgtttagctgctctgtgatgcatgaggccctgcacaatcattatacccagaagtccctgagcctgtctcccggcaagtga

SEQ ID NO: 61 - protein, 219 aa, Artificial Sequence
  Light chain of chimeric antibody 8F4
DVVMTQTAFSNPVTLGTSASISCRSSKSLLHSNGIIYLYWYLQKPGQSPQLLIYQMSNLASGVPDRFSSSGSGTDFTLRISRVEAEDVGVYYCAQNLELPFTFGSGTKLEIKRTVAAPSVFIFPPSDEQLKSGTASVVCLLNNFYPREAKVQWKVDNALQSGNSQESVTEQDSKDSTYSLSSTLTLSKADYEKHKVYACEVTHQGLSSPVTKSFNRGEC

SEQ ID NO: 62 - DNA, 660 bp, Artificial Sequence
  Light chain of chimeric antibody 8F4
gacgtggtcatgacccagacagccttctctaaccccgtgaccctgggcacatctgcttccatcagctgcagatccagcaagtctctgctgcactccaatggcatcatctacctgtattggtacctgcagaagcccggccagtcccctcagctgctgatctatcagatgagcaacctggcctctggcgtgccagaccgcttctcttccagcggctccggcaccgacttcaccctgaggatcagcagggtggaggctgaggatgtgggcgtgtactattgtgctcagaatctggagctgcccttcacctttggctccggcacaaagctggagatcaagcgtacggtggccgctcccagcgtgttcatctttcccccttctgacgagcagctgaagtctggcaccgcttccgtggtgtgcctgctgaacaatttctaccccagagaggccaaggtgcagtggaaggtggataacgctctgcagtccggcaatagccaggagtctgtgaccgagcaggactccaaggatagcacatattctctgtcttccaccctgacactgtctaaggccgactacgagaagcacaaggtgtatgcttgcgaggtgacccatcagggcctgagctctcctgtgacaaagtcctttaatcgcggcgagtgttga

SEQ ID NO: 63 - protein, 445 aa, Artificial Sequence
  Heavy chain of chimeric antibody 17E2
QVQLQQSGAELVRPGASVTLSCKASGYTFTDYEMHWVKQTPVLGLEWIGAIDPETGDTAYNQKFKGKATLTADKSSSTAYMELSSLASEDSAVYYCIRVDSNYDYFDYWGQDTTLTVSSASTKGPSVFPLAPCSRSTSESTAALGCLVKDYFPEPVTVSWNSGALTSGVHTFPAVLQSSGLYSLSSVVTVPSSNFGTQTYTCNVDHKPSNTKVDKTVERKCCVECPPCPAPPVAGPSVFLFPPKPKDTLMISRTPEVTCVVVDVSHEDPEVQFNWYVDGVEVHNAKTKPREEQFNSTFRVVSVLTVVHQDWLNGKEYKCKVSNKGLPAPIEKTISKTKGQPREPQVYTLPPSREEMTKNQVSLTCLVKGFYPSDISVEWESNGQPENNYKTTPPMLDSDGSFFLYSKLTVDKSRWQQGNVFSCSVMHEALHNHYTQKSLSLSPGK

SEQ ID NO: 64 - DNA, 1338 bp, Artificial Sequence
  Heavy chain of chimeric antibody 17E2
caggtgcagctgcagcagtccggagctgagctggtgaggccaggagcttccgtgaccctgagctgcaaggcctctggctacaccttcacagactatgagatgcactgggtgaagcagacacccgtgctgggactggagtggatcggagctatcgaccctgagaccggcgatacagcttacaaccagaagtttaagggcaaggccaccctgacagctgacaagtccagctctaccgcttatatggagctgtccagcctggccagcgaggactccgccgtgtactattgtatccgggtggatagcaattacgactatttcgattactggggccaggataccacactgacagtgtcttccgctagcacaaagggccctagcgtgttcccactggctccctgctccagaagcacatctgagtccaccgccgctctgggctgtctggtgaaggactacttccctgagccagtgacagtgtcctggaacagcggcgccctgacatccggagtgcacacctttccagctgtgctgcagtccagcggcctgtacagcctgtcttccgtggtgaccgtgcccagctctaattttggcacccagacatatacctgcaacgtggaccataagccttctaatacaaaggtggataagaccgtggagaggaagtgctgcgtggagtgcccaccttgtccagctccaccagtggctggcccttccgtgttcctgtttcctccaaagccaaaggacacactgatgatctctcggacacccgaggtgacctgcgtggtggtggacgtgtcccacgaggatccagaggtgcagttcaactggtacgtggatggcgtggaggtgcataatgccaagaccaagcccagggaggagcagttcaactctacatttcgggtggtgtccgtgctgaccgtggtgcaccaggattggctgaacggcaaggagtataagtgcaaggtgagcaataagggcctgcccgctcctatcgagaagacaatctctaagaccaagggccagcctagagagccacaggtgtacaccctgcccccttcccgcgaggagatgacaaagaaccaggtgagcctgacctgtctggtgaagggcttctatccttctgacatctccgtggagtgggagagcaatggccagccagagaacaattacaagaccacaccacccatgctggacagcgatggctctttctttctgtatagcaagctgacagtggataagtctcgctggcagcagggcaacgtgtttagctgctctgtgatgcatgaggccctgcacaatcattatacccagaagtccctgagcctgtctcccggcaagtga

SEQ ID NO: 65 - protein, 213 aa, Artificial Sequence
  Light chain of chimeric antibody 17E2
DIVLTQSPPILSASPGEKVTMTCRASSSVSYMHWYQQKPGSSPKPWIYDTSNLASGVPARFSGSGSGTSYSLTISRVEAEDAATYYCQQWSSNPLTFGAGTKLELKRTVAAPSVFIFPPSDEQLKSGTASVVCLLNNFYPREAKVQWKVDNALQSGNSQESVTEQDSKDSTYSLSSTLTLSKADYEKHKVYACEVTHQGLSSPVTKSFNRGEC

SEQ ID NO: 66 - DNA, 642 bp, Artificial Sequence
  Light chain of chimeric antibody 17E2
gacatcgtgctgacccagagcccacctatcctgagcgcctctccaggagagaaggtgaccatgacatgcagggcttccagctccgtgtcctacatgcactggtatcagcagaagcctggctccagcccaaagccctggatctacgacacctctaacctggcttccggagtgccagctaggttctccggcagcggctctggcacctcctatagcctgacaatctccagggtggaggctgaggatgctgctacatactattgtcagcagtggtcttccaatcctctgacctttggcgctggcacaaagctggagctgaagcgtacggtggccgctcccagcgtgttcatctttcccccttctgacgagcagctgaagtctggcaccgcttccgtggtgtgcctgctgaacaatttctaccccagagaggccaaggtgcagtggaaggtggataacgctctgcagtccggcaatagccaggagtctgtgaccgagcaggactccaaggatagcacatattctctgtcttccaccctgacactgtctaaggccgactacgagaagcacaaggtgtatgcttgcgaggtgacccatcagggcctgagctctcctgtgacaaagtcctttaatcgcggcgagtgttga

SEQ ID NO: 67 - protein, 444 aa, Artificial Sequence
  Heavy chain of chimeric antibody 31C8
QVQLQQSGPELVRPGASVTLSCKASGYIFIDSEMHWVKQTPVHGLEWIGAIDPETGDTVYNQKFKGKATLTADKSSSTASMELSSLTSEDSAVYYCTGSTTDYYFAYWGQGTTLTVSSASTKGPSVFPLAPCSRSTSESTAALGCLVKDYFPEPVTVSWNSGALTSGVHTFPAVLQSSGLYSLSSVVTVPSSNFGTQTYTCNVDHKPSNTKVDKTVERKCCVECPPCPAPPVAGPSVFLFPPKPKDTLMISRTPEVTCVVVDVSHEDPEVQFNWYVDGVEVHNAKTKPREEQFNSTFRVVSVLTVVHQDWLNGKEYKCKVSNKGLPAPIEKTISKTKGQPREPQVYTLPPSREEMTKNQVSLTCLVKGFYPSDISVEWESNGQPENNYKTTPPMLDSDGSFFLYSKLTVDKSRWQQGNVFSCSVMHEALHNHYTQKSLSLSPGK

SEQ ID NO: 68 - DNA, 1335 bp, Artificial Sequence
  Heavy chain of chimeric antibody 31C8
caggtgcagctgcagcagtctggaccagagctggtgaggcctggagcctccgtgaccctgagctgcaaggcttctggctacatcttcatcgactccgagatgcactgggtgaagcagacaccagtgcatggactggagtggatcggagctatcgacccagagaccggcgatacagtgtataaccagaagtttaagggcaaggccaccctgacagctgataagtccagctctaccgcctccatggagctgtccagcctgacaagcgaggactccgccgtgtactattgtaccggcagcaccacagattactatttcgcttactggggccagggcaccacactgacagtgtcttccgctagcacaaagggccctagcgtgttcccactggctccctgctccagaagcacatctgagtccaccgccgctctgggctgtctggtgaaggactacttccctgagccagtgacagtgtcctggaacagcggcgccctgacatccggagtgcacacctttccagctgtgctgcagtccagcggcctgtacagcctgtcttccgtggtgaccgtgcccagctctaattttggcacccagacatatacctgcaacgtggaccataagccttctaatacaaaggtggataagaccgtggagaggaagtgctgcgtggagtgcccaccttgtccagctccaccagtggctggcccttccgtgttcctgtttcctccaaagccaaaggacacactgatgatctctcggacacccgaggtgacctgcgtggtggtggacgtgtcccacgaggatccagaggtgcagttcaactggtacgtggatggcgtggaggtgcataatgccaagaccaagcccagggaggagcagttcaactctacatttcgggtggtgtccgtgctgaccgtggtgcaccaggattggctgaacggcaaggagtataagtgcaaggtgagcaataagggcctgcccgctcctatcgagaagacaatctctaagaccaagggccagcctagagagccacaggtgtacaccctgcccccttcccgcgaggagatgacaaagaaccaggtgagcctgacctgtctggtgaagggcttctatccttctgacatctccgtggagtgggagagcaatggccagccagagaacaattacaagaccacaccacccatgctggacagcgatggctctttctttctgtatagcaagctgacagtggataagtctcgctggcagcagggcaacgtgtttagctgctctgtgatgcatgaggccctgcacaatcattatacccagaagtccctgagcctgtctcccggcaagtga

SEQ ID NO: 69 - protein, 219 aa, Artificial Sequence; identical to SEQ ID NO: 57
  Light chain of chimeric antibody 31C8

SEQ ID NO: 70 - DNA, 660 bp, Artificial Sequence; identical to SEQ ID NO: 58
  Light chain of chimeric antibody 31C8

SEQ ID NO: 71 - protein, 118 aa, Artificial Sequence
  HV of humanized antibody 31C8-1.1
EVQLVQSGAEVKKPGATVKISCKASGYIFIDSEMHWVQQAPGKGLEWMGAIDPETGDTVYAEKFQGRVTITADKSSSTAYMELSSLRSEDTAVYYCTGSTTDYYFAYWGQGTLVTVSS

SEQ ID NO: 72 - DNA, 354 bp, Artificial Sequence
  HV of humanized antibody 31C8-1.1
gaggtgcagctggtgcagtctggcgccgaggtgaagaagccaggcgctaccgtgaagatcagctgcaaggcctctggctacatcttcatcgactccgagatgcactgggtgcagcaggctccaggcaagggactggagtggatgggcgctatcgaccctgagaccggcgatacagtgtacgctgagaagtttcagggcagggtgaccatcacagccgataagtccagctctacagcttatatggagctgtccagcctgcggtccgaggacaccgccgtgtactattgtacaggcagcaccacagattactatttcgcttattggggccagggcaccctggtgacagtgtcttcc

SEQ ID NO: 73 - protein, 118 aa, Artificial Sequence
  HV of humanized antibody 31C8-1.2
QVQLVQSGAKVKKPGATVKISCKASGYIFIDSEMHWVQQAPGKGLEWMGAIDPETGDTVYAKKFKGRVTITADKSSSTAYMELSSLRSEDTAVYYCTGSTTDYYFAYWGQGTLVTVSS

SEQ ID NO: 74 - DNA, 354 bp, Artificial Sequence
  HV of humanized antibody 31C8-1.2
caggtgcagctggtgcagtctggcgccaaggtgaagaagccaggcgctaccgtgaagatcagctgcaaggcctctggctacatcttcatcgactccgagatgcactgggtgcagcaggctccaggcaagggactggagtggatgggcgctatcgaccctgagaccggcgatacagtgtacgctaagaagtttaagggcagggtgaccatcacagccgataagtccagctctacagcttatatggagctgtccagcctgcggtccgaggacaccgccgtgtactattgtacaggcagcaccacagattactatttcgcttattggggccagggcaccctggtgacagtgtcttcc

SEQ ID NO: 75 - protein, 444 aa, Artificial Sequence
  Heavy chain of humanized antibody 31C8-1.1
EVQLVQSGAEVKKPGATVKISCKASGYIFIDSEMHWVQQAPGKGLEWMGAIDPETGDTVYAEKFQGRVTITADKSSSTAYMELSSLRSEDTAVYYCTGSTTDYYFAYWGQGTLVTVSSASTKGPSVFPLAPCSRSTSESTAALGCLVKDYFPEPVTVSWNSGALTSGVHTFPAVLQSSGLYSLSSVVTVPSSNFGTQTYTCNVDHKPSNTKVDKTVERKCCVECPPCPAPPVAGPSVFLFPPKPKDTLMISRTPEVTCVVVDVSHEDPEVQFNWYVDGVEVHNAKTKPREEQFNSTFRVVSVLTVVHQDWLNGKEYKCKVSNKGLPAPIEKTISKTKGQPREPQVYTLPPSREEMTKNQVSLTCLVKGFYPSDISVEWESNGQPENNYKTTPPMLDSDGSFFLYSKLTVDKSRWQQGNVFSCSVMHEALHNHYTQKSLSLSPGK

SEQ ID NO: 76 - DNA, 1335 bp, Artificial Sequence
  Heavy chain of humanized antibody 31C8-1.1
gaggtgcagctggtgcagtctggcgccgaggtgaagaagccaggcgctaccgtgaagatcagctgcaaggcctctggctacatcttcatcgactccgagatgcactgggtgcagcaggctccaggcaagggactggagtggatgggcgctatcgaccctgagaccggcgatacagtgtacgctgagaagtttcagggcagggtgaccatcacagccgataagtccagctctacagcttatatggagctgtccagcctgcggtccgaggacaccgccgtgtactattgtacaggcagcaccacagattactatttcgcttattggggccagggcaccctggtgacagtgtcttccgcctccaccaagggccctagcgtgttcccactggctccctgctccagaagcacatctgagtccaccgccgctctgggctgtctggtgaaggactacttccctgagccagtgacagtgtcctggaacagcggcgccctgacatccggagtgcacacctttccagctgtgctgcagtccagcggcctgtacagcctgtcttccgtggtgaccgtgcccagctctaattttggcacccagacatatacctgcaacgtggaccataagccttctaatacaaaggtggataagaccgtggagaggaagtgctgcgtggagtgcccaccttgtccagctccaccagtggctggcccttccgtgttcctgtttcctccaaagccaaaggacacactgatgatctctcggacacccgaggtgacctgcgtggtggtggacgtgtcccacgaggatccagaggtgcagttcaactggtacgtggatggcgtggaggtgcataatgccaagaccaagcccagggaggagcagttcaactctacatttcgggtggtgtccgtgctgaccgtggtgcaccaggattggctgaacggcaaggagtataagtgcaaggtgagcaataagggcctgcccgctcctatcgagaagacaatctctaagaccaagggccagcctagagagccacaggtgtacaccctgcccccttcccgcgaggagatgacaaagaaccaggtgagcctgacctgtctggtgaagggcttctatccttctgacatctccgtggagtgggagagcaatggccagccagagaacaattacaagaccacaccacccatgctggacagcgatggctctttctttctgtatagcaagctgacagtggataagtctcgctggcagcagggcaacgtgtttagctgctctgtgatgcatgaggccctgcacaatcattatacccagaagtccctgagcctgtctcccggcaagtga

SEQ ID NO: 77 - protein, 444 aa, Artificial Sequence
  Heavy chain of humanized antibody 31C8-1.2
QVQLVQSGAKVKKPGATVKISCKASGYIFIDSEMHWVQQAPGKGLEWMGAIDPETGDTVYAKKFKGRVTITADKSSSTAYMELSSLRSEDTAVYYCTGSTTDYYFAYWGQGTLVTVSSASTKGPSVFPLAPCSRSTSESTAALGCLVKDYFPEPVTVSWNSGALTSGVHTFPAVLQSSGLYSLSSVVTVPSSNFGTQTYTCNVDHKPSNTKVDKTVERKCCVECPPCPAPPVAGPSVFLFPPKPKDTLMISRTPEVTCVVVDVSHEDPEVQFNWYVDGVEVHNAKTKPREEQFNSTFRVVSVLTVVHQDWLNGKEYKCKVSNKGLPAPIEKTISKTKGQPREPQVYTLPPSREEMTKNQVSLTCLVKGFYPSDISVEWESNGQPENNYKTTPPMLDSDGSFFLYSKLTVDKSRWQQGNVFSCSVMHEALHNHYTQKSLSLSPGK

SEQ ID NO: 78 - DNA, 1335 bp, Artificial Sequence
  Heavy chain of humanized antibody 31C8-1.2
caggtgcagctggtgcagtctggcgccaaggtgaagaagccaggcgctaccgtgaagatcagctgcaaggcctctggctacatcttcatcgactccgagatgcactgggtgcagcaggctccaggcaagggactggagtggatgggcgctatcgaccctgagaccggcgatacagtgtacgctaagaagtttaagggcagggtgaccatcacagccgataagtccagctctacagcttatatggagctgtccagcctgcggtccgaggacaccgccgtgtactattgtacaggcagcaccacagattactatttcgcttattggggccagggcaccctggtgacagtgtcttccgcctccaccaagggccctagcgtgttcccactggctccctgctccagaagcacatctgagtccaccgccgctctgggctgtctggtgaaggactacttccctgagccagtgacagtgtcctggaacagcggcgccctgacatccggagtgcacacctttccagctgtgctgcagtccagcggcctgtacagcctgtcttccgtggtgaccgtgcccagctctaattttggcacccagacatatacctgcaacgtggaccataagccttctaatacaaaggtggataagaccgtggagaggaagtgctgcgtggagtgcccaccttgtccagctccaccagtggctggcccttccgtgttcctgtttcctccaaagccaaaggacacactgatgatctctcggacacccgaggtgacctgcgtggtggtggacgtgtcccacgaggatccagaggtgcagttcaactggtacgtggatggcgtggaggtgcataatgccaagaccaagcccagggaggagcagttcaactctacatttcgggtggtgtccgtgctgaccgtggtgcaccaggattggctgaacggcaaggagtataagtgcaaggtgagcaataagggcctgcccgctcctatcgagaagacaatctctaagaccaagggccagcctagagagccacaggtgtacaccctgcccccttcccgcgaggagatgacaaagaaccaggtgagcctgacctgtctggtgaagggcttctatccttctgacatctccgtggagtgggagagcaatggccagccagagaacaattacaagaccacaccacccatgctggacagcgatggctctttctttctgtatagcaagctgacagtggataagtctcgctggcagcagggcaacgtgtttagctgctctgtgatgcatgaggccctgcacaatcattatacccagaagtccctgagcctgtctcccggcaagtga

SEQ ID NO: 79 - protein, 112 aa, Artificial Sequence
  LVs of humanized antibodies 31C8-1.1 and 31C8-1.2
DIQMTQSPSSLSASVGDRVTITCRSSKSLLHSNGIIYLYWYQQKPGKAPKLLIYQLSNLASGVPSRFSSSGSGTDFTLTISSLQPEDFATYYCAQNLELPFTFGQGTKVEIK

SEQ ID NO: 80 - DNA, 336 bp, Artificial Sequence
  LVs of humanized antibodies 31C8-1.1 and 31C8-1.2
gacatccagatgacccagagcccttccagcctgtccgccagcgtgggcgatagggtgaccatcacatgccggtcttccaagtctctgctgcactccaacggcatcatctacctgtattggtaccagcagaagcccggcaaggcccctaagctgctgatctatcagctgagcaatctggcttctggcgtgccatccaggttcagctcttccggctctggcaccgactttaccctgacaatcagctctctgcagccagaggatttcgccacatactattgtgctcagaacctggagctgcccttcacctttggccagggcacaaaggtggagatcaag

SEQ ID NO: 81 - protein, 219 aa, Artificial Sequence
  Light chains of humanized antibodies 31C8-1.1 and 31C8-1.2
DIQMTQSPSSLSASVGDRVTITCRSSKSLLHSNGIIYLYWYQQKPGKAPKLLIYQLSNLASGVPSRFSSSGSGTDFTLTISSLQPEDFATYYCAQNLELPFTFGQGTKVEIKRTVAAPSVFIFPPSDEQLKSGTASVVCLLNNFYPREAKVQWKVDNALQSGNSQESVTEQDSKDSTYSLSSTLTLSKADYEKHKVYACEVTHQGLSSPVTKSFNRGEC

SEQ ID NO: 82 - DNA, 660 bp, Artificial Sequence
  Light chains of humanized antibodies 31C8-1.1 and 31C8-1.2
gacatccagatgacccagagcccttccagcctgtccgccagcgtgggcgatagggtgaccatcacatgccggtcttccaagtctctgctgcactccaacggcatcatctacctgtattggtaccagcagaagcccggcaaggcccctaagctgctgatctatcagctgagcaatctggcttctggcgtgccatccaggttcagctcttccggctctggcaccgactttaccctgacaatcagctctctgcagccagaggatttcgccacatactattgtgctcagaacctggagctgcccttcacctttggccagggcacaaaggtggagatcaagcgtacggtggccgctcccagcgtgttcatctttcccccttctgacgagcagctgaagtctggcaccgcttccgtggtgtgcctgctgaacaatttctaccccagagaggccaaggtgcagtggaaggtggataacgctctgcagtccggcaatagccaggagtctgtgaccgagcaggactccaaggatagcacatattctctgtcttccaccctgacactgtctaaggccgactacgagaagcacaaggtgtatgcttgcgaggtgacccatcagggcctgagctctcctgtgacaaagtcctttaatcgcggcgagtgttga

SEQ ID NO: 83 - protein, 447 aa, Artificial Sequence
  Heavy chain of RG6149
EVQLVQSGAEVKKPGESLKISCKGSGYSFTNYWIGWVRQMPGKGLEWMGIIYPGNSDTRFSPSFQGQVTISADKSITTAYLQWSSLKASDTAMYYCARHGTSSDYYGLDVWGQGTTVTVSSASTKGPSVFPLAPCSRSTSESTAALGCLVKDYFPEPVTVSWNSGALTSGVHTFPAVLQSSGLYSLSSVVTVPSSNFGTQTYTCNVDHKPSNTKVDKTVERKCCVECPPCPAPPVAGPSVFLFPPKPKDTLMISRTPEVTCVVVDVSHEDPEVQFNWYVDGVEVHNAKTKPREEQFNSTFRVVSVLTVVHQDWLNGKEYKCKVSNKGLPAPIEKTISKTKGQPREPQVYTLPPSREEMTKNQVSLTCLVKGFYPSDIAVEWESNGQPENNYKTTPPMLDSDGSFFLYSKLTVDKSRWQQGNVFSCSVMHEALHNHYTQKSLSLSPGK

SEQ ID NO: 84 - protein, 214 aa, Artificial Sequence
  Light chain of RG6149
DIQMTQSPSSLSASVGDRVTITCQASQDISNYLNWYQQKPGKAPKLLIYDASNLETGVPSRFSGSGSGTDFTFTISSLQPEDIATYYCQQDDNFPLTFGGGTKVEIKRTVAAPSVFIFPPSDEQLKSGTASVVCLLNNFYPREAKVQWKVDNALQSGNSQESVTEQDSKDSTYSLSSTLTLSKADYEKHKVYACEVTHQGLSSPVTKSFNRGEC

SEQ ID NO: 85 - protein, 449 aa, Artificial Sequence
  Heavy chain of GSK3772847
EVQLLESGGGLVQPGGSLRLSCAASGFTFSIYDMIWVRQAPGKGLEWVSSIRGEGGGTYYADSVKGRFTISRDNSKNTLYLQMNSLRAEDTAVYYCARDPWSTEGSFFVLDYWGQGTLVTVSSASTKGPSVFPLAPCSRSTSESTAALGCLVKDYFPEPVTVSWNSGALTSGVHTFPAVLQSSGLYSLSSVVTVTSSNFGTQTYTCNVDHKPSNTKVDKTVERKCCVECPPCPAPPAAASSVFLFPPKPKDTLMISRTPEVTCVVVDVSAEDPEVQFNWYVDGVEVHNAKTKPREEQFNSTFRVVSVLTVLHQDWLNGKEYKCKVSNKGLPSSIEKTISKTKGQPREPQVYTLPPSREEMTKNQVSLTCLVKGFYPSDIAVEWESNGQPENNYKTTPPMLDSDGSFFLYSKLTVDKSRWQQGNVFSCSVMHEALHNHYTQKSLSLSPGK

SEQ ID NO: 86 - protein, 214 aa, Artificial Sequence
  Light chain of GSK3772847
EIVLTQSPATLSLSPGERATLSCRASQSVDDDLAWYQQKPGQAPRLLIYDASNRATGIPARFSGSGSGTDFTLTISSLEPEDFAVYYCQQYITAPLTFGQGTKVEIKRTVAAPSVFIFPPSDEQLKSGTASVVCLLNNFYPREAKVQWKVDNALQSGNSQESVTEQDSKDSTYSLSSTLTLSKADYEKHKVYACEVTHQGLSSPVTKSFNRGEC